European Patent Specification EP 3 801 580 B1, published August 30, 2023. Title: Nouvelle utilisation extrait bactérien AV13. Applicant: PIERRE FABRE DERMO-COSMETIQUE. The sequence listing filed with the application follows.

SEQUENCE LISTING (2 sequences)

SEQ ID NO: 1 - DNA, 1487 bp, artificial
  Nouvelle bactérie LMB64, classe des beta-proteobacteria, issue d'une nappe phréatique
agtttgatcatggctcagattgaacgcgggcggcatgctttacacatgcaagtcgaacggcagcacgggcttcggcctggtggcgagtggcgaacgggtgagtaatgcgtcggaacgcgccgagtagtgggggataacgcagcgaaagctgtgctaataccgcatacgtactgaggtagaaagtgggggaccttcgggcctcacgctattcgagcggccgacgtctgattagctagttggtggggtaaaggcccaccaaggcgacgatcagtagcgggtctgagaggatgatccgccacactgggactgagacacggcccagactcctacgggaggcagcagtggggaattttggacaatgggcgcaagcctgatccagccatgccgcgtgtctgaagaaggccttcgggttgtaaaggacttttgtccgggagcaaagcctgcttgttaataccgagtggggatgagagtaccggaagaataagcaccggctaactacgtgccagcagccgcggtaatacgtagggtgcaagcgttaatcggaattactgggcgtaaagcgtgcgcaggcggttgtgcaagtctgatgtgaaagccccgggctcaacctgggaacggcattggagactgcacggctagagtgcgtcagaggggggtagaattccacgtgtagcagtgaaatgcgtagagatgtggaggaataccgatggcgaaggcagccccctgggatgacactgacgctcatgcacgaaagcgtggggagcaaacaggattagataccctggtagtccacgccctaaacgatgtcaattagctgttgggggtttgaatccttggtagcgaagctaacgcgtgaaattgaccgcctggggagtacggccgcaaggttaaaactcaaaggaattgacggggacccgcacaagcggtggatgatgtggattaattcgatgcaacgcgaaaaaccttacctgctcttgacatgtaccgaagcctgaagagatttgggtgtgcccgaaagggagcggtaacacaggtgctgcatggctgtcgtcagctcgtgtcgtgagatgttgggttaagtcccgcaacgagcgcaacccttgtcattagttgccatcatttggttgggcactctaatgagactgccggtgacaaaccggaggaaggtggggatgacgtcaagtcctcatggcccttatgagcagggcttcacacgtcatacaatggtcggtacagagggtcgccaagccgcgaggtggagccaatctcagaaagccgatcgtagtccggatcgcactctgcaactcgagtgcgtgaagtcggaatcgctagtaatcgcagatcagcatgctgcggtgaatacgttcccgggtcttgtacacaccgcccgtcacaccatgggagtgggggataccagaagtgggtaggctaaccgcaagggaggccgcttaccacggtatgcttcatgactggggtgaagtcgtaac

SEQ ID NO: 2 - DNA, 10948 bp, artificial
  Nouvelle bactérie LMB64, classe des beta-proteobacteria, issue d'une nappe phréatique
gggcgcagcaccatcgcccaggccaaaagccacccgtgccgattcggcggcctgttgctcgcgctcaatgcgctgcgcctggtcggccaagtcggcggcttgctgctcggccttgcccgccagggtgtcacgctcgcgggtcagttccgccacctgctcggctagggcatcgcgctcggcctcgatcacctcaccagcggccgccagctcggcggcttcgctctgcgcctggaccaagcggccctcgacctcggcgcgggcctgggcggctgcgcgctcgatctcggcggcaatggcggcggtcaatgcctggggcagttccggcgcagcagcagcggccaccggccgggcctctcgccaggcagttagatgcttgtgaacggtattcgggctgccggtgcccaaacgctcgcggatcgcgcggatagtcggctgctgcccttcgccgaccagcgcatcagcggcggcggcgaacgggtggcccgtgcagaggcccgcgtcgagcagatcgagcagcaggccgccaaggcggcacaggcccacgaagaagcccgcgccgccgccacgcaggaagcccggcaagtgcaagccgaacgcgacgaagcccgcaaggtggccgccgaggcgcgcgagcagaccgcgcgcctggctgggcaactcgaagccctcaccgcgaaggagcgaaaagccgatgaaagaccgtgaccacaacgaagcgatggccggcatgtttcaggccgacccccgatttgccgccgactatctgcgccaggtgttggccgatggcgagcctaccgacgtgcgcgccggcttgcggcaaatggcggatgtgctgcgcgtcagtcaggccgccgcgccgaccgattctgcgccttcggcgggcctctttgaccgggccggcgtgcgctacgaagtggcgtgcgatgtgatcggggcgttgattgcccattacgccgaaatcatgggacgggaacgcgagcaggcgcagccgaatgaggcggttttgcgcgtggccggagccatgaaggcggcgctggccggggagcgggatgatctcgatccgcgcgatagcgccggcatcgaggcggcgatttcgcgctatgcgccactggcgcgccggctgtatggccaggctgaaaacgaccacgcccgccaggaacagcgtcgcgccgatttcgaccaggtgcatgcttcgctggccttggaggggctggccatgagcgcggacgatttggcggttcaggcgctgctgatccggggcgacattacccacgatgaggcggtgcagtgctaccgcatcctgcatcgccatgcgcggtaaaaccgactggccgcccgaggtggccggtgtgctgggtttgctcgaatcgcagccgccagaggcggcgatgctggtgggctgttttctggcggcggtagcccatcccgatcatgcggccgaattggcgatgttcgacaaattgccgccagcggcccggatggtcgtcgggcgatttttcctcgtttttctggcgggcggcctggacgatgccgggcgcgaaaaactgcattcgcacatgcaggcatggtttgtccgtcagcgccgttttcggtgaatggcttgcctcatccactagggccgggcaaggggtgaacagcgggcgatgctggcttgcgggacgaccccgcacccccggaaaacttgtcacacaccacgcaactcccgttgcttcgctaaaagccttgtgccgcaaggcttttagcgaggcgacaccgaagacacatcgcggcgacaccgaaagggccgaaccggcctaaaacccttgctgcgcaaggagaacagccgcgctttcgcgcgcgaaagtgcttcaaatgcctgtcggcatcagcagggtatggatcggcacgccgaaggcgttggcgatgcgctccaggttgtccaaggagatgtttctgacttggcgctcgcagtgcgcaacgaaggtgcgatgtaggccgcactcaaaggcgagcgcttcttgtgaccagcctctttcccggcgtaatcggatcatgttggccgcgagcacggcccgcgcggaatgcgcggttggtgcgggaggttgagcggcgggagacatgcaaaccagtctcctgatatgccgcttttacgtcagccgtgtttaagtcacaatatggttttctcatagagaaagacggcgtgacgatgggcagaaaaacagcaatcaggcgagggggtgccgtgttggccagcctgttgatttgcgcaattgaaccggtcggcgcggcctccctggtcggcggtcaaaccgatgattccgtgtgcgacctgggcagcgcgccacagaacgcccggaagctgtcggcagcgggcgacttcatccgcgcgcagtgcaaaaacggtcaaatgttggtgggttccggcatcgtgcctgccggcgggtttgactcggaagtggtgcgcctggcgcgcaccttctgccgcatggcggacattcagactcggcgcacgcagggcaacatggccggcctcgtcatggagatcgacgaggtacggtgcatcatcgggaagttgccgacatgagaaaagcgatgttggctggctttctggccgttgtggtggccaacgtggttgccgctgagggcggtgcgcccttgcgcggcggtgtttgcatcggaccgttccgtggcgctgattccgtcgtgcactgcgagcacatcggcaaggtgacgatccgccagatttacgaaaagggctttcgggtcgttcacatgcaggacgacaagaacacagccagctacgttgtgctggttatcgaggagcaggcgcgatgagggcgaaagcgtggcggatgctgtttgccgggcggcgctgggtgctctggcttcccgtgccggcgtcggtatggctggcactgcccgaatggcagcacattcccgccatgttgttgggcggcctgatcgtgtggattcccttctggctcgcgtggtggctcagtgatggcttcgcgggcatgtccaggtggccaggaaccggcgcacctgcggtatctggcggggtgaacccgcacaccggcaagccatgcacggtgtatcaccagccgtggggagataccttcgtgggtggagactgattatttgattgaggaacgatgacaagggccagcaacaagctggcccttgtcgttttctggactgttttacccacaacatccgctctgctgctgaattggcggacatggcaccgagccgaacgaacagaacacgcagcaatcccccggcttggggcgcagcagcgtatggcaggccgggcactcgtagtagaactggcaggcgtccgtgggcatggtttcctgctgtgcgtggccgcagtgcgggcaggtcagcacggattcgagaatgacggcgctcatcgtggcgttacctctgcacggtggacggatagcctgcgttcgtcgttgccgaggtcaacgcttccggcttggccttgtcggcgtcataggtgacggtggccgttttcttgtcgaaatcgaccttgacggcgctcacaccgggcactttctccagcgacttcttgactgtgatcgggcatagctcgcaggtcatgttctgaacggccagcgtgacggttttcggggtggcggccagcacggcgagcggcacggcagccagcagagcaatcagcagtttgcgcatgggagtctcctttcaatagaacagcggggcgaaccacggcacggccaacagggcaagcaacagcacagtgacgatccagaacgtcaggcgctgccgctggcgtgtgcgcggatcagcgcatggcgtgccgggcgtgcagacctgcggcaccagatagagcttgcggaaggccagtccgagaaagagcagcgtcatgccgatgaaaaagggccggtacggctccatcgcggtcaggctgccaacccatgagccaccaatgccaagcaccagcaggacaagcggcccgacacagcacaccgacgcgccgatggcggtcagtacgctcacgatcaacgagcttttttcagtgagtcgtgccatgtcgctttccttgtacctgtttgcccaagtgttactctaaatcccgtacctaagtacggagtcaagggggtgtgatgggaacagaactgaccatcggcaagctggctgacgctgccggggtgaatatcgagacgattcgctactaccagcggcgcggcctgctggatgagccgcctaaaccgccaggggggcatcggcgctatgcgcctgagcaggcaaaacgtgtgcgatttatcaagcgggcacaggcgcttggtttcacgctggacgaggtaggcgcgctactgaccctggatgcggcctgcgcctgcggtgagacgcgagcgctggctgtgcgcaagctgggtctgatcgagcagaagatggctgacctcgcggccatgcggcaggcgctgggtggattggtgcagcagtgtgatgcgggcgacggtggagccagctgtcccatcatcgacgtgctggcaggtaattagatgtgttcaaaaaatggtggttttctggacacatgccggtttgccctgtcctgagttgtcctgatgcgttaaagtgttcatttattcgttcagctttcaatgtggcggaactgttcatgaatcaacgcatcggctatgcccgcgtttcgaccgacgaccaaaacctagacctgcaacgggacgcactccggcaggctggatgctcaaccatttacgaggaagcagccagcggaaagagcgcagcaaggcccgagcttgagcagtgtcggaaggctctccggcccggcgacacgcttgtggtgtggcggcttgatcgccttgggcgcagcctgcccgacctggtgcagatcgtggctgatcttgaacagcgcggcgtgcatttcgagagcctgaccgagaagatcgagacggggagcgcagcgggtaagctgcaattccatgttttcgctgcactcgccgagttcgagcgcggcctgatccgggagcgaacccgggcagggctggatgcagctcgcgcccgtggccgatccggtggacgcaaaccgaagctggacgccaagcagatacgccacattaaggcgctactacgtgacccgaatacctgtgttgctgaactcgcccgtgactacggcgtgtcgagaacaactatctataaacactgcggtgtggttctgccgcgtacagccgatgaaggggcaatatgacaaaaaagacaacagcattcgatgtattcgagaaatgcgtccaagcagttcaggctggtgaactgatcgaatccgtttctgcgaaggacaaggaattccatttccagaactggtttcagaagcgcctccagagcctgtcgatgcacttcgaggggtcgggtcgcaacacctacccggacttctgcttggtagagcacaccgagggctacgagatcaagggtttggcatggcctggccgcgagcgcgactacgactcgaacagccaagtgccgactggctatcacaacggccgtcaaatcttctacgtgttcgggcgctaccccgcagacctgtctggctatgccgatcagggcaacggccgcaggcagtacccggtggttgacctcgtggtctgccacggcgacttcctcaacgccgatcacaactacgtccataagaacaagagcgtaaagggctttggcacctacggcgacatcatgatccgcgaccggaagatgtacgtcgcgccgacgccatttgcgctgaccgaaggcaccactggcctgatgactttgatcctgccggagaacttcggcaccgatgaccgttaccaggtggtcggtaacctcactcgcgtcgaggcggaaacgctggtggttggctacaactttgacctgcgcacgaacgagctgagcgcagagcgcgtgcccaatcccaacgcaggcacccagcaccgattcgtggcctaccggctcaaggatcaagcgagcaagcctgtctccatgactggcacccaggtgcagcccgacgagaacaacctgccggacgacgaatgaacaccatcaccgacaagatcgggttcgcttacccggttgcagcgaccgcgctggagtgcgacttcccgctggtcgaaatcagccagatcgccgagcaggaaagttggcgaaaggagatcaacaggccgatctaccacatccacaagtggtgggcgaccagacttgggtcggtgtttcgtggcattacccttggtgctttgagtcagcctggtactgacctctgggcgcagttctacaaaacgcacgacctggccggtaaggtagtgctcgatcccttcatgggcagtggcacgacgcttggcgaggccgtcaagctgggtgccaaggccatcggctgcgacatcaacccagtcagtaccttcctcgtacgtcaggcgttcacgccggcgtccgaggcagagctgcgtgccgctttcgagcggctggaacgtgacgtggcaccggagattcggcgctactaccagacgcgcgatcctaagacgggcgagctgattcaggtcttgtactacttctgggtcaagacggtgacgacgcccgagggcgaggtaatccccttgctgtcgcgctacgtgttttcacaagacgcctacccgaagaagaagccgcgagcgcagatcgtgtgccctggctgctggagtgtgctggaggatcgctacgatgcgactgacctgcactgccagcactgcggccaccagttcaatccgcaggaaggcccggccgctggtcagtacgtcaaaaccaagggcggtcaccgttaccgcatcaaggaactactgccaaaggacggtacgccgccctctcatcgaatgtacgcgatgatggccttgcgagcggatggatcgaaggtctatctgccggtgcggaatgaggacttggccctctacgaggaagcccaagaacgccttgctacagaggcactgccgctgccgaaaacctctgttcgacctggccacaacaccgaccaggcgcgcggctacaactacacccaatggcgcgacttcttcaatgcgcgccaactgctgtgccttggcctgctgctgcgggaaatcctgaccatcgacgacctggcagtgcaagagcagatgctgtgcttgttctccagcaccttggagttcaacaacctgttttgcagcttcaagggtgagggaacaggggccgtgcggcatatgttctcgaaccacatcctcaagccagagcgcaccccgctggagaactccgtgtggggcactggcaagagcagcggtacgtttagcacgttgttcgagtctcgcctgctacgtgcgaagcgctacctcgatgagccgttcgagatcgcgttcgagcatgaccaggacggtaaccgcgcaggctcgcgcaagacggtggctagccatccgatccgcgcccgtcgcgtcgaaacctggccggaattggaggccgcagatcatggcctgctgatcctcaacggtgacagctcgaagctgccggtgcccgctggttcggtggatgccgtggtgactgatccgccctacttcgacttcgttcattactcggagttgagcgacttcttttttgcttggctcacccctgtgctgcgccagcgctatccgtggatggcccgcgaggactcgtctgaccaaggggaggtgcagcacaaagaccctcgtgtgttcgcccgtcagcttgcgtcggtgttcacggaggcgtgccgcgtgcttaaggacgatggagtgttggcgttcagcttccaccactcgcgtgccgagggctgggcggccatctatgaagcgatcaacaaggcgggcctggccgtagttgcggctcaccctgtccatgccgagctgcgcgcggcaagtcccaagactgcggccaaagacccgatcagccttgatgcgattctggtgtgtcgcaaaaaggcgtttgccctgcaccagtcgcctgctatccaggatgtccgccaggctgttgatgcgctggcatcacggctgcaagctgctggccttcgcatctcggcgggtgaccgcttcgtgatcggcgcagcgcaaaccttgattgcacgcgctgctgatgacatgggcttcgacgagatcaaggttgatcttgaggcaattcggctggccgtggggccaagggctgcaacatcaaaggctgcgagtgcgtgggatgacgatgtgcccttctgattggctgcacggccttgtcggcgcatgcgttttgatggcagccgctgcacgcaagccgcgtccctccgcgtaaagttcatttatacgcaaatacgtatttgcgtgatacaataacgccatattaatggaggtgcgtaaatgcggactattgttgtggctagccaaaaaggtggcgtcggcaagacaacgattgcaggtcacttgggtgtcatggccgagcagagcaaagaggggccagtggcgctgatcgacacagacccacaaggctcgctcgcgtcctggtggaatgagcgaaccaatgaggcaccgctgtttgcacgggtggaaatcggcaagctgaccgagcaccttcaggcattgtccaagggtggcatcaagctggccatcatcgacaccccgccctctgttacggaaatgattcagcaggtgctccgcaccgccgacttggtactgatccccaccaggccgagtccgcatgacttgcgcgcggtcggatctaccgtcgaactggtggagaacgcaggcaagcgaatgatcttcgtcatcaatggggcggcacctcgcgcgcggatcgcgggtgaggctgccgtggcgctttcgcagcatggcacggttgcccccgtgacgctgtaccagcgcaccgacttcgccagctcgatgatcgacggccgcaccgtccaggaaatcgaccccaaggggcggtcggccgaagaaatcgggcagttgtggaaatacgtatctacacaactgcgtaaaatttgatataatacgtacatgcgtattaatggagatacgtaaatggctaaaactgcatctttgactgccggcctggtggccaagaaaggggaggcgtcccctgctacggttgtcgcggcaccccaggttcaacctatcgaagtgaaggcatcggcgactggcggcggccgggattactacaaggcgttgaccgtcaagttggatcgtgaccgctacgagagtctgaaaagcatgggcgtgaagctggacaagaagagccaggaaatctttgtcgaggccctggatttgtggatgaagtcggccgctggccagcaacacgcctaagaggcccctatgcgttcagtgcgctctgccgtcgaactcgccaaggagttggccgaaaaagccaaggcccgccgcctagcggcggaaaagaacgagctgggacttgaaggcccggcgcagggcaacgccggcaccactcccagcccggtgaaggttgcggccgaagtggtgggcgagcagccggcacgacgcaagggagcgccgaaagggccgcgtggcctgatgccggtgcatcatccaaaccgcgatttcttcttgtgcgatctgtttgactacgccctaaaggatgacggcgtgagcatggaggcccccatcttcaccttggcaaccaggccggacacctctgtttggcattgggaaagcaaggatgggacacgcgccatcaccgtcacgccaagcgtgaaggggagggccacgcagtttgataaggatttacttatttacgtagttagccagatgaccgaggctatcaatcgcggtcggcctgatgcgaacaatcgaaccgtgcgctttcgcgtctatgactacttggtctcaaccaacaagccgactggcggcaaggagtaccagcgactggaggatgccctagacaggctgcggggtacatcgatcaagacgaacatcaagacgggtggccagcgtgtgaaggaaggcttcggcatcgtcgatagctggacgatcatcgagaaggcccccgacgatgaccgcatgattgccgtcgaggtcacgctctccaagtggcttttcaatgcagtgcaggcccacgaggttctgaccatcaacccggactatttccggctgcgtaagccaattgagcgccgtttgtacgagctggccaggaagcactgtggcgaccaggccttttttgtgattgggctggaactgttgcaggacaagtgcggcagcaagtcggcactgttcgagttccgccgtgccttgcgcgagatcatcaaggccgacaccttgccagactaccgcatgacgcttgatgacgagaaagaccaggtgattttctacacccgcgacacgaagaagctagcggcgtctaccgctctggcccggcgcttccagtgacgcccaaagtattgacggtcaatacttcgttatttcacccatgcggtgttaccgctgcgtgttggacgttcccttgacctagcggccgaggcagggctttcgcgctttgcattgagccaccaagtgcgtctcgctccttcgagcatcaagccctaacgcgtttcatgtcactttcgcgcacgaaagtcgaggcaagaggcttgatcgtgtctatcgttacatcacccatgcctgtggatggacacgttacatcacccatgttttctgtggatgggcacgttacatcacccatacctcacttcgttacatcgcccatgcagcgatttgtggaagccttgagcagcaaggctttacgagcgttatccacagccgtaacacgcgcgcgcgattttttaactttataaatctttaacgcggttgcggacaaagcccgcgccgcctcttgggggctacgcccccgccggctcctacgggccgcaagcggccctccgcccgcgcttcgcgctccctcccggcatccccgaggggtttcgcttcgctgcacccctcgcgcttcgcgctcacccgcatatcgaggcccccaaagggggccggatggtgccccc